European Patent Application EP 4 166 658 A1, published April 19, 2023. Title: Diatom-based genetic engineering system methodology for the eco-sustainable production of ovothiols. Applicant: Stazione Zoologica Anton Dohrn. Application EP. The sequence listing filed with the application follows.

SEQUENCE LISTING (18 sequences)

SEQ ID NO: 1 - DNA, 22 bp, synthetic construct
  source 1..22: mol_type = other DNA
tctagaggtcaagtccagactc

SEQ ID NO: 2 - DNA, 44 bp, synthetic construct
  source 1..44: mol_type = other DNA
caggagtctggacttgacctctagaggtaccccgctttggtttc

SEQ ID NO: 3 - DNA, 34 bp, synthetic construct
  misc_feature 1..34: note = Lhcf2p_rev
  source 1..34: mol_type = other DNA
gtggagagagcatcatcttgacttctggcaaccg

SEQ ID NO: 4 - DNA, 32 bp, synthetic construct
  source 1..32: mol_type = other DNA
gccagaagtcaagatgatgctctctccacaag

SEQ ID NO: 5 - DNA, 31 bp, synthetic construct
  source 1..31: mol_type = other DNA
ccttgctcaccattcctgtcttacgccaacc

SEQ ID NO: 6 - DNA, 31 bp, synthetic construct
  source 1..31: mol_type = other DNA
gcgtaagacaggaatggtgagcaagggcgag

SEQ ID NO: 7 - DNA, 49 bp, synthetic construct
  source 1..49: mol_type = other DNA
caagcttgcatgcctgcaggtcgacgctgaagacgagctagtgttattc

SEQ ID NO: 8 - DNA, 18 bp, synthetic construct
  source 1..18: mol_type = other DNA
gtcgacctgcaggcatgc

SEQ ID NO: 9 - DNA, 20 bp, synthetic construct
  misc_feature 1..20: note = Lhcf2pfw2
  source 1..20: mol_type = other DNA
cgccgtaaacagcaaatcct

SEQ ID NO: 10 - DNA, 20 bp, synthetic construct
  source 1..20: mol_type = other DNA
aaggaaggaaagtcggcagg

SEQ ID NO: 11 - DNA, 22 bp, synthetic construct
  source 1..22: mol_type = other DNA
gaattcatggtgagcaagggcg

SEQ ID NO: 12 - DNA, 24 bp, synthetic construct
  source 1..24: mol_type = other DNA
gaattcgatatcaagcttatcgat

SEQ ID NO: 13 - DNA, 60 bp, synthetic construct
  source 1..60: mol_type = other DNA
aagtcaagtcgacggtatcgataagcttgatatcgaattcatgatgctctctccacaagc

SEQ ID NO: 14 - DNA, 40 bp
ccaaagtcgaggtagttgtttcatcctgtcttacgccaac

SEQ ID NO: 15 - DNA, 20 bp, synthetic construct
  source 1..20: mol_type = other DNA
cgccgtaaacagcaaatcct

SEQ ID NO: 16 - DNA, 20 bp, synthetic construct
  source 1..20: mol_type = other DNA
aactccagcaggaccatgtg

SEQ ID NO: 17 - protein, 933 aa, synthetic construct
MMLSPQAARMGTVCTTLRKIVSTARQRSLSHSAFASVRSETAFGARAFSTRAKSTLAALEDSDDEDLTFRSQGHAAAAAALSKAGLNKSHDEAWMINVNRNDDNEWLNGPRSAEWFTGIHPSQCPGADQAGTIRSLSLPNLSAVTREAAKEYFDNSWTLYETLFAGLKGEEGFYRPPVHGLRHPQIFYYGHTACLYINKLRVSKVLPKPVNAYFESIFEVGVDEMLWDDMNKNDMLWPTVSEVHEYRQQVYKTVVDAILNHPSLDQRNGPVKVDQDHPMWALFMGFEHERIHMETSSVLFRETPYHLVQTPQHWPPIHPSAFNDASPTSNPIETLDYPANRMIAVDNGTVDLGKPADFPSFGWDNEYGERNMDVPPFFASEHMITNGEYWQFVDNGGYRNREYWCDDGWAWRSHRNLKWPFFWEPAGPAGSNKFSLRTIFKIVPMPWSWPVDVNYYEAQAFCRWKTEKEGSPTSKPYRILTEAEHHIIRNHDHNLEAARRDVSADKVMVTSGQAFPKGSAGSNLNLAFSSQNPVDFFEPSQTGHRDTTGSAWEWTEDHFNPLKGFEVHHVYDDFSTPCFDGKHSIIVGGSFISTGDEASVFARFHFRPHFLQHSGFRLVASDHDAPATHLFAGNFDGQVAARDAAVAQEESKPRQSSLGSGSGSGNVYETDDSLHMYLGLHYPNSGEKEGVAPILPHDNSPNHGTGFPQRVAGLLSSLKPEFNNNRALDIGCAVGGASFELAKTFDHVDAFDFSGSFVSAAKRMQSAENIKFRVPVEAELYEDLQAIHEHGVTDSVRSKVQFFTGDACRLIDMKEDGILGSYDGVVMSNLLCRLPDPMACLAGLPEIINPGGVVVMVTPFSWLTEFTPRGKWLGGFYDPVTNEAIYSKDILRQIMASNGFEKIHEVQMPLVIREHQRKYQYIVSEATGWRKTG

SEQ ID NO: 18 - DNA, 2802 bp, synthetic construct
  source 1..2802: mol_type = other DNA
atgatgctctctccacaagccgcccgtatgggtaccgtgtgcacgacactccgcaagatagtttcgacggcgcgtcagcggtctctctcgcattcggcgttcgcgtcggtccgtagcgagaccgcgtttggagcccgggcgttttcgacgcgtgcgaaatctactctagcggcactcgaagactcggatgacgaggatctcacctttcgtagtcagggacacgccgcagccgccgcggctttgagcaaggcaggattgaacaagtctcacgatgaggcctggatgatcaacgtcaatcgcaacgacgacaacgaatggctgaacgggccgcgcagtgccgaatggtttacgggcattcaccctagtcaatgtcctggagccgaccaagcgggcaccatccgctcgctttcacttccgaatctgtcggccgttacccgtgaagctgcaaaagaatactttgacaactcatggacgctctacgagacattgtttgccggtctcaaaggagaagaaggattttatcgcccgccagtccacggtctccgccacccccagatattctactacggacacactgcttgtctctacatcaacaagctccgcgtcagtaaagtcttacccaaacctgtgaacgcctatttcgagtccatcttcgaagtcggtgtagacgaaatgctctgggatgacatgaacaagaatgatatgctttggcccacagtttcggaggtgcacgagtatcgacagcaagtatacaaaacggttgtggacgctattttgaatcatcctagtcttgatcaaaggaacggtccagtgaaagtcgatcaggatcatccaatgtgggcattgttcatgggcttcgaacacgagcggatccatatggaaacgagttcagtcttgttccgtgagacgccgtaccatttggtccaaacaccccagcattggcctccgattcatccgtcggctttcaacgatgcctcgcccacaagcaatccgatagaaactttggattaccccgcgaaccgcatgattgccgtggacaatggaaccgtcgatctcggaaagcctgccgactttccttcctttggatgggacaatgagtacggtgaacgcaatatggatgtgcctccattcttcgctagtgaacacatgatcacaaatggagaatactggcagtttgtcgacaatggtggctatcgaaatcgagagtattggtgcgacgacggctgggcgtggcgcagtcatcgcaatcttaagtggccttttttttgggagcccgcaggacccgctgggtccaataagttttcgttgcgaaccattttcaagatcgttcccatgccgtggagttggcctgttgatgtaaattactacgaagcgcaagccttctgtcgatggaagaccgagaaagaaggatctccgacttcaaaaccgtatagaattctcaccgaagcggagcatcacatcattcgaaaccacgatcacaacttggaggctgctcgtagagacgtttcggcggataaggtgatggtgacttcagggcaagcgtttcccaaaggatcggctggatcaaatttgaacctggcattctctagccaaaaccccgtcgatttctttgagccgtcccaaactggccaccgtgataccaccggaagtgcctgggaatggacggaagaccacttcaaccctttaaagggatttgaagtccaccacgtgtacgatgatttttccactccatgttttgatggcaagcactctatcattgtggggggatcttttataagtactggcgacgaggcatcagtttttgcacgattccatttccgaccccatttcctacaacattctggtttccgtctggttgcatcagatcacgatgctcctgctacgcacctttttgccggaaatttcgatggtcaagttgccgcacgcgatgccgcggtcgcgcaggaagaatccaagccgagacagtcttcattaggaagcggcagtggcagcggcaatgtttacgagacggatgacagcttgcatatgtatcttggccttcattaccctaattctggcgagaaggaaggcgttgccccgatccttcctcacgacaactctccaaaccatggaactggcttcccgcaacgagtggcaggtcttctgtcctcactgaaacccgagttcaataacaatcgcgcattggatattggctgtgctgttggaggggcgtcttttgaacttgctaagactttcgatcacgtggacgcctttgatttcagtggatctttcgtgagcgctgccaagcgaatgcaatcggcagaaaatatcaagtttcgggttcccgtggaggctgaactatatgaagaccttcaggctatccacgaacatggtgtgacggattcggtgcgctccaaagtgcagttctttacaggggacgcctgccgactcatcgatatgaaagaagacggaattcttggctcatatgatggcgtggtcatgtcgaatttactctgccgcctcccagatccaatggcatgcctcgccggacttccagagattataaatcccggtggagtggtcgtgatggtgacgccattttcgtggttgactgagttcaccccccggggcaaatggctaggaggattttacgaccccgtaacaaacgaagctatctattcgaaggacatcctgcgccaaattatggcctcgaatgggttcgagaagattcatgaggttcagatgccgctcgtcattcgggagcaccaacgtaaataccagtatattgtcagcgaagctacaggttggcgtaagacaggatga